European Patent Application EP 4 700 389 A1, published February 25, 2026. Title: Asbestos Detection. Applicant: Université de Liège. Application EP. The sequence listing filed with the application follows.

SEQUENCE LISTING (1 sequence)

SEQ ID NO: 1 - protein, 12 aa, Bacteriophage M13
TGAAEVAMMSKR